European Patent Application EP 4 227 410 A1, published August 16, 2023. Title: A method for producing allulose using a novel allulose-producing enzyme. Applicant: AMANO ENZYME INC. The sequence listing filed with the application follows.

SEQUENCE LISTING (6 sequences)

SEQ ID NO: 1 - DNA, 23 bp, Artificial
  Primer
atgaacaagctyggaytscaygc

SEQ ID NO: 2 - DNA, 24 bp, Artificial
  Primer
tcagcgsttrtggcgyccyagcgc

SEQ ID NO: 3 - DNA, 21 bp, Artificial
  Primer
atccatatctgcagtcaagcc

SEQ ID NO: 4 - DNA, 21 bp, Artificial
  Primer
tcgatttcccgagcatattcc

SEQ ID NO: 5 - DNA, 882 bp, Asaia krungthepensis
atgaacaagctcggactccacgcttttgtctggactgctggctggacgcctgaagacgccgccatggccatccgctcgacggctgaactcggctacgatctgatcgaggcctcgaccatggacctcaaggccttcgacgtgcccgcaacactgcgcgaactcgaagccaatcgtctcgggatcaccatgtccttcggcttgactgcagatatggatatctcctcgggcgacccggagcgtatccgtcggggagaggcgcatctgctcgatgccatttcccttgcccgagatgtcggggcgacccatgtctgcggcattctctattccgccttccagaaatacgcgacgccggtgacggcagaaggcgtgcgcggctctatcgaagtggtgcgtcgtgtcgctgaaaaggcgcaggccagtggcatcacgctgggcatggaagtggtcaatcgctacgagtccaacgtgctcaatacggcacgtcaggcgattgcctatgtgaagcgcgtcgagatgcccaatgtgaagctgcacctcgattgctatcacatgaatatcgaagaagcggattccgccgaggccattcgcgaggcgggcgatctgctgggctatttccataccggggattcgcatcgcggctatcttggatcgggttcggtcgatttcccgagcatattccgcgcgctggagagcattcagtatcaagggccgatcactttcgaatccttctcctcagcggtggtcggtcaaccgctcgaagggattctgggcatttggcgcaatctctgggaagacagccgtgatctcgcggcccatgccaaggccttcaccgatgtgcagatgaaatcggcacgcgaggcgctcggccgccagaagcgctaa

SEQ ID NO: 6 - protein, 293 aa, Asaia krungthepensis
MNKLGLHAFVWTAGWTPEDAAMAIRSTAELGYDLIEASTMDLKAFDVPATLRELEANRLGITMSFGLTADMDISSGDPERIRRGEAHLLDAISLARDVGATHVCGILYSAFQKYATPVTAEGVRGSIEVVRRVAEKAQASGITLGMEVVNRYESNVLNTARQAIAYVKRVEMPNVKLHLDCYHMNIEEADSAEAIREAGDLLGYFHTGDSHRGYLGSGSVDFPSIFRALESIQYQGPITFESFSSAVVGQPLEGILGIWRNLWEDSRDLAAHAKAFTDVQMKSAREALGRQKR